European Patent Application EP 4 549 556 A1, published May 7, 2025. Title: Method for generation of endocannabinoid receptor gene knockout microglia cells. Applicant: VILNIUS UNIVERSITY. Application EP. The sequence listing filed with the application follows.

SEQUENCE LISTING (14 sequences)

SEQ ID NO: 1 - RNA, 24 nt, synthetic construct
  source 1..24: mol_type = other RNA
accggcccacgtagaggaggtctg

SEQ ID NO: 2 - RNA, 24 nt, synthetic construct
  source 1..24: mol_type = other RNA
aaaccagacctcctctacgtgggc

SEQ ID NO: 3 - RNA, 24 nt, synthetic construct
  source 1..24: mol_type = other RNA
accgattcagtacgaagatatcaa

SEQ ID NO: 4 - RNA, 24 nt, synthetic construct
  source 1..24: mol_type = other RNA
aaacttgatatcttcgtactgaat

SEQ ID NO: 5 - RNA, 24 nt, synthetic construct
  source 1..24: mol_type = other RNA
accgaagttagagggaatttctgt

SEQ ID NO: 6 - RNA, 24 nt, synthetic construct
  source 1..24: mol_type = other RNA
aaacacagaaattccctctaactt

SEQ ID NO: 7 - RNA, 24 nt, synthetic construct
  source 1..24: mol_type = other RNA
accgtcccttccaagaaaagatga

SEQ ID NO: 8 - RNA, 25 nt, synthetic construct
  source 1..25: mol_type = other RNA
aaactcatcttttcttggaagggac

SEQ ID NO: 9 - RNA, 24 nt, synthetic construct
  source 1..24: mol_type = other RNA
accgttggaagggactacccctga

SEQ ID NO: 10 - RNA, 24 nt, synthetic construct
  source 1..24: mol_type = other RNA
aaactcaggggtagtcccttccaa

SEQ ID NO: 11 - RNA, 24 nt, synthetic construct
  source 1..24: mol_type = other RNA
accgggcaggagacaactccccgt

SEQ ID NO: 12 - RNA, 24 nt, synthetic construct
  source 1..24: mol_type = other RNA
aaacacggggagttgtctcctgcc

SEQ ID NO: 13 - RNA, 24 nt, synthetic construct
  source 1..24: mol_type = other RNA
accgggatcatgtactccttcatg

SEQ ID NO: 14 - RNA, 24 nt, synthetic construct
  source 1..24: mol_type = other RNA
aaaccatgaaggagtacatgatcc